European Patent Application EP 4 814 007 A1, published September 30, 2026. Title: ENGINEERED ANTIBODY CH3 DOMAINS. Applicant: Merck Patent GmbH. Application EP, filed March 27, 2025. The sequence listing filed with the application follows.

SEQUENCE LISTING (103 sequences)

SEQ ID NO: 1 - protein, 99 aa, synthetic construct
  VARIANT 37: note = X at position 37 is I or V
  VARIANT 38: note = X at position 38 is A or L
  VARIANT 42: note = X at position 42 is L or E
GQPFRPEVHLLPPSREEMTKNQVSLTCLARGFYPKDXXVRWXSNSQEENNYKTTPSRQEPSQGTTTFAVTSKLTVDKSRWQQGNVFSCMVGHEALPLAF

SEQ ID NO: 2 - protein, 126 aa, synthetic construct
  VARIANT 37: note = X at position 37 is I or V
  VARIANT 38: note = X at position 38 is A or L
  VARIANT 42: note = X at position 42 is L or E
GQPFRPEVHLLPPSREEMTKNQVSLTCLARGFYPKDXXVRWXSNSQEENNYKTTPSRQEPSQGTTTFAVTSKLTVDKSRWQQGNVFSCMVGHEALPLAFTQKTISLSPGKPTHVNVSVVMAEVDGT

SEQ ID NO: 3 - protein, 99 aa, synthetic construct
  VARIANT 42: note = X at position 42 is L or E
GQPFRPEVHLLPPSREEMTKNQVSLTCLARGFYPKDIAVRWXSNSQEENNYKTTPSRQEPSQGTTTFAVTSKLTVDKSRWQQGNVFSCMVGHEALPLAF

SEQ ID NO: 4 - protein, 126 aa, synthetic construct
  VARIANT 42: note = X at position 42 is L or E
GQPFRPEVHLLPPSREEMTKNQVSLTCLARGFYPKDIAVRWXSNSQEENNYKTTPSRQEPSQGTTTFAVTSKLTVDKSRWQQGNVFSCMVGHEALPLAFTQKTISLSPGKPTHVNVSVVMAEVDGT

SEQ ID NO: 5 - protein, 99 aa, synthetic construct
GQPFRPEVHLLPPSREEMTKNQVSLTCLARGFYPKDIAVRWLSNSQEENNYKTTPSRQEPSQGTTTFAVTSKLTVDKSRWQQGNVFSCMVGHEALPLAF

SEQ ID NO: 6 - protein, 126 aa, synthetic construct
GQPFRPEVHLLPPSREEMTKNQVSLTCLARGFYPKDIAVRWLSNSQEENNYKTTPSRQEPSQGTTTFAVTSKLTVDKSRWQQGNVFSCMVGHEALPLAFTQKTISLSPGKPTHVNVSVVMAEVDGT

SEQ ID NO: 7 - protein, 99 aa, synthetic construct
GQPFRPEVHLLPPSREEMTKNQVSLTCLARGFYPKDIAVRWESNSQEENNYKTTPSRQEPSQGTTTFAVTSKLTVDKSRWQQGNVFSCMVGHEALPLAF

SEQ ID NO: 8 - protein, 126 aa, synthetic construct
GQPFRPEVHLLPPSREEMTKNQVSLTCLARGFYPKDIAVRWESNSQEENNYKTTPSRQEPSQGTTTFAVTSKLTVDKSRWQQGNVFSCMVGHEALPLAFTQKTISLSPGKPTHVNVSVVMAEVDGT

SEQ ID NO: 9 - protein, 99 aa, synthetic construct
GQPFRPEVHLLPPSREEMTKNQVSLTCLARGFYPKDVLVRWESNSQEENNYKTTPSRQEPSQGTTTFAVTSKLTVDKSRWQQGNVFSCMVGHEALPLAF

SEQ ID NO: 10 - protein, 126 aa, synthetic construct
GQPFRPEVHLLPPSREEMTKNQVSLTCLARGFYPKDVLVRWESNSQEENNYKTTPSRQEPSQGTTTFAVTSKLTVDKSRWQQGNVFSCMVGHEALPLAFTQKTISLSPGKPTHVNVSVVMAEVDGT

SEQ ID NO: 11 - protein, 99 aa, synthetic construct
GQPFRPEVHLLPPSREEMTKNQVSLTCLARGFYPKDVLVRWLSNSQEENNYKTTPSRQEPSQGTTTFAVTSKLTVDKSRWQQGNVFSCMVGHEALPLAF

SEQ ID NO: 12 - protein, 126 aa, synthetic construct
GQPFRPEVHLLPPSREEMTKNQVSLTCLARGFYPKDVLVRWLSNSQEENNYKTTPSRQEPSQGTTTFAVTSKLTVDKSRWQQGNVFSCMVGHEALPLAFTQKTISLSPGKPTHVNVSVVMAEVDGT

SEQ ID NO: 13 - protein, 99 aa, synthetic construct; identical to SEQ ID NO: 1
  VARIANT 37: note = X at position 37 is I or V
  VARIANT 38: note = X at position 38 is A or L
  VARIANT 42: note = X at position 42 is L or E

SEQ ID NO: 14 - protein, 126 aa, synthetic construct; identical to SEQ ID NO: 2
  VARIANT 37: note = X at position 37 is I or V
  VARIANT 38: note = X at position 38 is A or L

SEQ ID NO: 15 - protein, 99 aa, synthetic construct; identical to SEQ ID NO: 3
  VARIANT 42: note = X at position 42 is L or E

SEQ ID NO: 16 - protein, 126 aa, synthetic construct; identical to SEQ ID NO: 4
  VARIANT 42: note = X at position 42 is L or E

SEQ ID NO: 17 - protein, 99 aa, synthetic construct; identical to SEQ ID NO: 5

SEQ ID NO: 18 - protein, 126 aa, synthetic construct; identical to SEQ ID NO: 6

SEQ ID NO: 19 - protein, 99 aa, synthetic construct; identical to SEQ ID NO: 7

SEQ ID NO: 20 - protein, 126 aa, synthetic construct; identical to SEQ ID NO: 8

SEQ ID NO: 21 - protein, 99 aa, synthetic construct; identical to SEQ ID NO: 9

SEQ ID NO: 22 - protein, 126 aa, synthetic construct; identical to SEQ ID NO: 10

SEQ ID NO: 23 - protein, 99 aa, synthetic construct; identical to SEQ ID NO: 11

SEQ ID NO: 24 - protein, 126 aa, synthetic construct; identical to SEQ ID NO: 12

SEQ ID NO: 25 - protein, 99 aa, synthetic construct
  VARIANT 28: note = X at position 38 is I or V
  VARIANT 39: note = X at position 39 is A or L
GQPREPQVYTLPPPSEELALNELVTLTCLVKGFYPSDXXVRWLQGSQELPREKYLTWAPVLDSDGSFFLYSILRVAAEDWKKGDTFSCMVGHEALPLAF

SEQ ID NO: 26 - protein, 127 aa, synthetic construct
  VARIANT 38: note = X at position 38 is I or V
  VARIANT 39: note = X at position 39 is A or L
GQPREPQVYTLPPPSEELALNELVTLTCLVKGFYPSDXXVRWLQGSQELPREKYLTWAPVLDSDGSFFLYSILRVAAEDWKKGDTFSCMVGHEALPLAFTTQKSLDRSPGKPTHVNVSVVMAEVDGT

SEQ ID NO: 27 - protein, 99 aa, synthetic construct
GQPREPQVYTLPPPSEELALNELVTLTCLVKGFYPSDVLVRWLQGSQELPREKYLTWAPVLDSDGSFFLYSILRVAAEDWKKGDTFSCMVGHEALPLAF

SEQ ID NO: 28 - protein, 126 aa, synthetic construct
GQPREPQVYTLPPPSEELALNELVTLTCLVKGFYPSDVLVRWLQGSQELPREKYLTWAPVLDSDGSFFLYSILRVAAEDWKKGDTFSCMVGHEALPLAFTQKSLDRSPGKPTHVNVSVVMAEVDGT

SEQ ID NO: 29 - protein, 99 aa, synthetic construct
GQPREPQVYTLPPPSEELALNELVTLTCLVKGFYPSDIAVRWLQGSQELPREKYLTWAPVLDSDGSFFLYSILRVAAEDWKKGDTFSCMVGHEALPLAF

SEQ ID NO: 30 - protein, 126 aa, synthetic construct
GQPREPQVYTLPPPSEELALNELVTLTCLVKGFYPSDIAVRWLQGSQELPREKYLTWAPVLDSDGSFFLYSILRVAAEDWKKGDTFSCMVGHEALPLAFTQKSLDRSPGKPTHVNVSVVMAEVDGT

SEQ ID NO: 31 - protein, 99 aa, synthetic construct; identical to SEQ ID NO: 25
  VARIANT 38: note = X at position 38 is V or I
  VARIANT 39: note = X at position 39 is L or A

SEQ ID NO: 32 - protein, 126 aa, synthetic construct
  VARIANT 38: note = X at position 38 is V or I
  VARIANT 39: note = X at position 39 is L or A
GQPREPQVYTLPPPSEELALNELVTLTCLVKGFYPSDXXVRWLQGSQELPREKYLTWAPVLDSDGSFFLYSILRVAAEDWKKGDTFSCMVGHEALPLAFTQKSLDRSPGKPTHVNVSVVMAEVDGT

SEQ ID NO: 33 - protein, 99 aa, synthetic construct; identical to SEQ ID NO: 27

SEQ ID NO: 34 - protein, 126 aa, synthetic construct; identical to SEQ ID NO: 28

SEQ ID NO: 35 - protein, 99 aa, synthetic construct; identical to SEQ ID NO: 29

SEQ ID NO: 36 - protein, 126 aa, synthetic construct; identical to SEQ ID NO: 30

SEQ ID NO: 37 - protein, 126 aa, synthetic construct
GQPFRPEVHLLPPSREEMTKNQVSLTCLARGFYPKDIAVEWESNGQPENNYKTTPSRQEPSQGTTTFAVTSKLTVDKSRWQQGNVFSCSVMHEALHNHYTQKTISLSPGKPTHVNVSVVMAEVDGT

SEQ ID NO: 38 - protein, 126 aa, synthetic construct
GQPREPQVYTLPPPSEELALNELVTLTCLVKGFYPSDIAVEWLQGSQELPREKYLTWAPVLDSDGSFFLYSILRVAAEDWKKGDTFSCSVMHEALHNHYTQKSLDRSPGKPTHVNVSVVMAEVDGT

SEQ ID NO: 39 - protein, 126 aa, synthetic construct; identical to SEQ ID NO: 37

SEQ ID NO: 40 - protein, 126 aa, synthetic construct; identical to SEQ ID NO: 38

SEQ ID NO: 41 - protein, 101 aa, Homo sapiens
CCHPRLSLHRPALEDLLLGSEANLTCTLTGLRDASGVTFTWTPSSGKSAVQGPPERDLCGCYSVSSVLPGCAEPWNHGKTFTCTAAYPESKTPLTATLSKS

SEQ ID NO: 42 - protein, 129 aa, Homo sapiens
GNTFRPEVHLLPPPSEELALNELVTLTCLARGFSPKDVLVRWLQGSQELPREKYLTWASRQEPSQGTTTFAVTSILRVAAEDWKKGETFSCMVGHEALPLAFTQKTIDRLAGKPTHVNVSVVMAEVDGT

SEQ ID NO: 43 - protein, 101 aa, Homo sapiens; identical to SEQ ID NO: 41

SEQ ID NO: 44 - protein, 101 aa, Homo sapiens
CCHPRLSLHRPALEDLLLGSEANLTCTLTGLRDASGATFTWTPSSGKSAVQGPPERDLCGCYSVSSVLPGCAQPWNHGETFTCTAAHPELKTPLTANITKS

SEQ ID NO: 45 - protein, 110 aa, Homo sapiens
APELLGGPSVFLFPPKPKDTLMISRTPEVTCVVVDVSHEDPEVKFNWYVDGVEVHNAKTKPREEQYNSTYRVVSVLTVLHQDWLNGKEYKCKVSNKALPAPIEKTISKAK

SEQ ID NO: 46 - protein, 109 aa, Homo sapiens
APPVAGPSVFLFPPKPKDTLMISRTPEVTCVVVDVSHEDPEVQFNWYVDGVEVHNAKTKPREEQFNSTFRVVSVLTVVHQDWLNGKEYKCKVSNKGLPAPIEKTISKTK

SEQ ID NO: 47 - protein, 110 aa, Homo sapiens
APELLGGPSVFLFPPKPKDTLMISRTPEVTCVVVDVSHEDPEVQFKWYVDGVEVHNAKTKPREEQYNSTFRVVSVLTVLHQDWLNGKEYKCKVSNKALPAPIEKTISKTK

SEQ ID NO: 48 - protein, 110 aa, Homo sapiens
APEFLGGPSVFLFPPKPKDTLMISRTPEVTCVVVDVSQEDPEVQFNWYVDGVEVHNAKTKPREEQFNSTYRVVSVLTVLHQDWLNGKEYKCKVSNKGLPSSIEKTISKAK

SEQ ID NO: 49 - protein, 227 aa, synthetic construct
CCHPRLSLHRPALEDLLLGSEANLTCTLTGLRDASGVTFTWTPSSGKSAVQGPPERDLCGCYSVSSVLPGCAEPWNHGKTFTCTAAYPESKTPLTATLSKSGQPFRPEVHLLPPSREEMTKNQVSLTCLARGFYPKDIAVRWLSNSQEENNYKTTPSRQEPSQGTTTFAVTSKLTVDKSRWQQGNVFSCMVGHEALPLAFTQKTISLSPGKPTHVNVSVVMAEVDGT

SEQ ID NO: 50 - protein, 227 aa, synthetic construct
CCHPRLSLHRPALEDLLLGSEANLTCTLTGLRDASGVTFTWTPSSGKSAVQGPPERDLCGCYSVSSVLPGCAEPWNHGKTFTCTAAYPESKTPLTATLSKSGQPFRPEVHLLPPSREEMTKNQVSLTCLARGFYPKDVLVRWESNSQEENNYKTTPSRQEPSQGTTTFAVTSKLTVDKSRWQQGNVFSCMVGHEALPLAFTQKTISLSPGKPTHVNVSVVMAEVDGT

SEQ ID NO: 51 - protein, 226 aa, synthetic construct
CHPRLSLHRPALEDLLLGSEANLTCTLTGLRDASGVTFTWTPSSGKSAVQGPPERDLCGCYSVSSVLPGCAEPWNHGKTFTCTAAYPESKTPLTATLSKSGQPFRPEVHLLPPSREEMTKNQVSLTCLARGFYPKDIAVRWESNSQEENNYKTTPSRQEPSQGTTTFAVTSKLTVDKSRWQQGNVFSCMVGHEALPLAFTQKTISLSPGKPTHVNVSVVMAEVDGT

SEQ ID NO: 52 - protein, 227 aa, synthetic construct
CCHPRLSLHRPALEDLLLGSEANLTCTLTGLRDASGVTFTWTPSSGKSAVQGPPERDLCGCYSVSSVLPGCAEPWNHGKTFTCTAAYPESKTPLTATLSKSGQPFRPEVHLLPPSREEMTKNQVSLTCLARGFYPKDVLVRWLSNSQEENNYKTTPSRQEPSQGTTTFAVTSKLTVDKSRWQQGNVFSCMVGHEALPLAFTQKTISLSPGKPTHVNVSVVMAEVDGT

SEQ ID NO: 53 - protein, 227 aa, synthetic construct
CCHPRLSLHRPALEDLLLGSEANLTCTLTGLRDASGATFTWTPSSGKSAVQGPPERDLCGCYSVSSVLPGCAQPWNHGETFTCTAAHPELKTPLTANITKSGQPFRPEVHLLPPSREEMTKNQVSLTCLARGFYPKDIAVRWLSNSQEENNYKTTPSRQEPSQGTTTFAVTSKLTVDKSRWQQGNVFSCMVGHEALPLAFTQKTISLSPGKPTHVNVSVVMAEVDGT

SEQ ID NO: 54 - protein, 227 aa, synthetic construct
CCHPRLSLHRPALEDLLLGSEANLTCTLTGLRDASGVTFTWTPSSGKSAVQGPPERDLCGCYSVSSVLPGCAEPWNHGKTFTCTAAYPESKTPLTATLSKSGQPREPQVYTLPPPSEELALNELVTLTCLVKGFYPSDVLVRWLQGSQELPREKYLTWAPVLDSDGSFFLYSILRVAAEDWKKGDTFSCMVGHEALPLAFTQKSLDRSPGKPTHVNVSVVMAEVDGT

SEQ ID NO: 55 - protein, 227 aa, synthetic construct
CCHPRLSLHRPALEDLLLGSEANLTCTLTGLRDASGVTFTWTPSSGKSAVQGPPERDLCGCYSVSSVLPGCAEPWNHGKTFTCTAAYPESKTPLTATLSKSGQPREPQVYTLPPPSEELALNELVTLTCLVKGFYPSDIAVRWLQGSQELPREKYLTWAPVLDSDGSFFLYSILRVAAEDWKKGDTFSCMVGHEALPLAFTQKSLDRSPGKPTHVNVSVVMAEVDGT

SEQ ID NO: 56 - protein, 227 aa, synthetic construct
CCHPRLSLHRPALEDLLLGSEANLTCTLTGLRDASGATFTWTPSSGKSAVQGPPERDLCGCYSVSSVLPGCAQPWNHGETFTCTAAHPELKTPLTANITKSGQPREPQVYTLPPPSEELALNELVTLTCLVKGFYPSDVLVRWLQGSQELPREKYLTWAPVLDSDGSFFLYSILRVAAEDWKKGDTFSCMVGHEALPLAFTQKSLDRSPGKPTHVNVSVVMAEVDGT

SEQ ID NO: 57 - protein, 19 aa, Homo sapiens
VPSTPPTPSPSTPPTPSPS

SEQ ID NO: 58 - protein, 6 aa, Homo sapiens
VPPPPP

SEQ ID NO: 59 - protein, 470 aa, synthetic construct
EVQLVQSGAEVKKPGASVKVSCKASGFSLTNYGVHWMRQAPGQGLEWIGVIWSGGNTDYNTPFTSRVTITSDKSTSTAYMELSSLRSEDTAVYYCARALTYYDYEFAYWGQGTLVTVSSASPTSPKVFPLSLCSTQPDGNVVIACLVQGFFPQEPLSVTWSESGQGVTARNFPPSQDASGDLYTTSSQLTLPATQCLAGKSVTCHVKHYTNPSQDVTVPCPVPSTPPTPSPSTPPTPSPSCCHPRLSLHRPALEDLLLGSEANLTCTLTGLRDASGVTFTWTPSSGKSAVQGPPERDLCGCYSVSSVLPGCAEPWNHGKTFTCTAAYPESKTPLTATLSKSGNTFRPEVHLLPPPSEELALNELVTLTCLARGFSPKDVLVRWLQGSQELPREKYLTWASRQEPSQGTTTFAVTSILRVAAEDWKKGETFSCMVGHEALPLAFTQKTIDRLAGKPTHVNVSVVMAEVDGT

SEQ ID NO: 60 - protein, 214 aa, synthetic construct
DIQMTQSPSSLSASVGDRVTITCRASQSIGTNIHWYQQKPGKAPKLLIKYASESISGVPSRFSGSGYGTDFTLTISSLQPEDVATYYCQQNNNWPTTFGQGTKVEIKRTVAAPSVFIFPPSDEQLKSGTASVVCLLNNFYPREAKVQWKVDNALQSGNSQESVTEQDSKDSTYSLSSTLTLSKADYEKHKVYACEVTHQGLSSPVTKSFNRGEC

SEQ ID NO: 61 - protein, 490 aa, synthetic construct
EIVLTQSPATLSLSPGERATLSCRASQSVSSYLAWYQQKPGQAPRLLIYDASNRATGIPARFSGSGSGTDFTLTISSLEPEDFAVYYCQQRSNWPPSTFGQGTRLEIKGGGGSGGGGSGGGGSGGGGSEVQLLESGGGLVQPGGSLRLSCAASGFTFTSYAMSWVRQAPGKGLEWVSTISGSGGGTYYTDSVKGRFTISRDNSKNTLYLQMNSLRAEDTAVYYCAQGSSIFDYWGQGTLVTVSSVPSTPPTPSPSTPPTPSPSCCHPRLSLHRPALEDLLLGSEANLTCTLTGLRDASGVTFTWTPSSGKSAVQGPPERDLCGCYSVSSVLPGCAEPWNHGKTFTCTAAYPESKTPLTATLSKSGQPFRPEVHLLPPSREEMTKNQVSLTCLARGFYPKDIAVEWESNGQPENNYKTTPSRQEPSQGTTTFAVTSKLTVDKSRWQQGNVFSCSVMHEALHNHYTQKTISLSPGKPTHVNVSVVMAEVDGT

SEQ ID NO: 62 - protein, 467 aa, synthetic construct
EVQLVQSGAEVKKPGASVKVSCKASGFSLTNYGVHWMRQAPGQGLEWIGVIWSGGNTDYNTPFTSRVTITSDKSTSTAYMELSSLRSEDTAVYYCARALTYYDYEFAYWGQGTLVTVSSASPTSPKVFPLSLCSTQPDGNVVIACLVQGFFPQEPLSVTWSESGQGVTARNFPPSQDASGDLYTTSSQLTLPATQCLAGKSVTCHVKHYTNPSQDVTVPCPVPSTPPTPSPSTPPTPSPSCCHPRLSLHRPALEDLLLGSEANLTCTLTGLRDASGVTFTWTPSSGKSAVQGPPERDLCGCYSVSSVLPGCAEPWNHGKTFTCTAAYPESKTPLTATLSKSGQPREPQVYTLPPPSEELALNELVTLTCLVKGFYPSDIAVEWLQGSQELPREKYLTWAPVLDSDGSFFLYSILRVAAEDWKKGDTFSCSVMHEALHNHYTQKSLDRSPGKPTHVNVSVVMAEVDGT

SEQ ID NO: 63 - protein, 214 aa, synthetic construct; identical to SEQ ID NO: 60

SEQ ID NO: 64 - protein, 490 aa, synthetic construct
EIVLTQSPATLSLSPGERATLSCRASQSVSSYLAWYQQKPGQAPRLLIYDASNRATGIPARFSGSGSGTDFTLTISSLEPEDFAVYYCQQRSNWPPSTFGQGTRLEIKGGGGSGGGGSGGGGSGGGGSEVQLLESGGGLVQPGGSLRLSCAASGFTFTSYAMSWVRQAPGKGLEWVSTISGSGGGTYYTDSVKGRFTISRDNSKNTLYLQMNSLRAEDTAVYYCAQGSSIFDYWGQGTLVTVSSVPSTPPTPSPSTPPTPSPSCCHPRLSLHRPALEDLLLGSEANLTCTLTGLRDASGVTFTWTPSSGKSAVQGPPERDLCGCYSVSSVLPGCAEPWNHGKTFTCTAAYPESKTPLTATLSKSGQPFRPEVHLLPPSREEMTKNQVSLTCLARGFYPKDIAVRWESNSQEENNYKTTPSRQEPSQGTTTFAVTSKLTVDKSRWQQGNVFSCMVGHEALPLAFTQKTISLSPGKPTHVNVSVVMAEVDGT

SEQ ID NO: 65 - protein, 467 aa, synthetic construct
EVQLVQSGAEVKKPGASVKVSCKASGFSLTNYGVHWMRQAPGQGLEWIGVIWSGGNTDYNTPFTSRVTITSDKSTSTAYMELSSLRSEDTAVYYCARALTYYDYEFAYWGQGTLVTVSSASPTSPKVFPLSLCSTQPDGNVVIACLVQGFFPQEPLSVTWSESGQGVTARNFPPSQDASGDLYTTSSQLTLPATQCLAGKSVTCHVKHYTNPSQDVTVPCPVPSTPPTPSPSTPPTPSPSCCHPRLSLHRPALEDLLLGSEANLTCTLTGLRDASGVTFTWTPSSGKSAVQGPPERDLCGCYSVSSVLPGCAEPWNHGKTFTCTAAYPESKTPLTATLSKSGQPREPQVYTLPPPSEELALNELVTLTCLVKGFYPSDIAVRWLQGSQELPREKYLTWAPVLDSDGSFFLYSILRVAAEDWKKGDTFSCMVGHEALPLAFTQKSLDRSPGKPTHVNVSVVMAEVDGT

SEQ ID NO: 66 - protein, 214 aa, synthetic construct; identical to SEQ ID NO: 60

SEQ ID NO: 67 - protein, 491 aa, synthetic construct
EIVLTQSPATLSLSPGERATLSCRASQSVSSYLAWYQQKPGQAPRLLIYDASNRATGIPARFSGSGSGTDFTLTISSLEPEDFAVYYCQQRSNWPPSTFGQGTRLEIKGGGGSGGGGSGGGGSGGGGSEVQLLESGGGLVQPGGSLRLSCAASGFTFTSYAMSWVRQAPGKGLEWVSTISGSGGGTYYTDSVKGRFTISRDNSKNTLYLQMNSLRAEDTAVYYCAQGSSIFDYWGQGTLVTVSSVPSTPPTPSPSTPPTPSPSCCHPRLSLHRPALEDLLLGSEANLTCTLTGLRDASGVTFTWTPSSGKSAVQGPPERDLCGCYSVSSVLPGCAEPWNHGKTFTCTAAYPESKTPLTATLSKSGQPFRPEVHLLPPSREEMTKNQVSLTCLARGFYPKDIAVRWLSNSQEENNYKTTPSRQEPSQGTTTFAVTSKLTVDKSRWQQGNVFSCMVGHEALPLAFTQKTISLSPGKPTHVNVSVVMAEVDGTS

SEQ ID NO: 68 - protein, 467 aa, synthetic construct; identical to SEQ ID NO: 65

SEQ ID NO: 69 - protein, 214 aa, synthetic construct; identical to SEQ ID NO: 60

SEQ ID NO: 70 - protein, 490 aa, synthetic construct
EIVLTQSPATLSLSPGERATLSCRASQSVSSYLAWYQQKPGQAPRLLIYDASNRATGIPARFSGSGSGTDFTLTISSLEPEDFAVYYCQQRSNWPPSTFGQGTRLEIKGGGGSGGGGSGGGGSGGGGSEVQLLESGGGLVQPGGSLRLSCAASGFTFTSYAMSWVRQAPGKGLEWVSTISGSGGGTYYTDSVKGRFTISRDNSKNTLYLQMNSLRAEDTAVYYCAQGSSIFDYWGQGTLVTVSSVPSTPPTPSPSTPPTPSPSCCHPRLSLHRPALEDLLLGSEANLTCTLTGLRDASGVTFTWTPSSGKSAVQGPPERDLCGCYSVSSVLPGCAEPWNHGKTFTCTAAYPESKTPLTATLSKSGQPFRPEVHLLPPSREEMTKNQVSLTCLARGFYPKDIAVRWLSNSQEENNYKTTPSRQEPSQGTTTFAVTSKLTVDKSRWQQGNVFSCMVGHEALPLAFTQKTISLSPGKPTHVNVSVVMAEVDGT

SEQ ID NO: 71 - protein, 467 aa, synthetic construct
EVQLVQSGAEVKKPGASVKVSCKASGFSLTNYGVHWMRQAPGQGLEWIGVIWSGGNTDYNTPFTSRVTITSDKSTSTAYMELSSLRSEDTAVYYCARALTYYDYEFAYWGQGTLVTVSSASPTSPKVFPLSLCSTQPDGNVVIACLVQGFFPQEPLSVTWSESGQGVTARNFPPSQDASGDLYTTSSQLTLPATQCLAGKSVTCHVKHYTNPSQDVTVPCPVPSTPPTPSPSTPPTPSPSCCHPRLSLHRPALEDLLLGSEANLTCTLTGLRDASGVTFTWTPSSGKSAVQGPPERDLCGCYSVSSVLPGCAEPWNHGKTFTCTAAYPESKTPLTATLSKSGQPREPQVYTLPPPSEELALNELVTLTCLVKGFYPSDVLVRWLQGSQELPREKYLTWAPVLDSDGSFFLYSILRVAAEDWKKGDTFSCMVGHEALPLAFTQKSLDRSPGKPTHVNVSVVMAEVDGT

SEQ ID NO: 72 - protein, 214 aa, synthetic construct; identical to SEQ ID NO: 60

SEQ ID NO: 73 - protein, 490 aa, synthetic construct
EIVLTQSPATLSLSPGERATLSCRASQSVSSYLAWYQQKPGQAPRLLIYDASNRATGIPARFSGSGSGTDFTLTISSLEPEDFAVYYCQQRSNWPPSTFGQGTRLEIKGGGGSGGGGSGGGGSGGGGSEVQLLESGGGLVQPGGSLRLSCAASGFTFTSYAMSWVRQAPGKGLEWVSTISGSGGGTYYTDSVKGRFTISRDNSKNTLYLQMNSLRAEDTAVYYCAQGSSIFDYWGQGTLVTVSSVPSTPPTPSPSTPPTPSPSCCHPRLSLHRPALEDLLLGSEANLTCTLTGLRDASGVTFTWTPSSGKSAVQGPPERDLCGCYSVSSVLPGCAEPWNHGKTFTCTAAYPESKTPLTATLSKSGQPFRPEVHLLPPSREEMTKNQVSLTCLARGFYPKDVLVRWESNSQEENNYKTTPSRQEPSQGTTTFAVTSKLTVDKSRWQQGNVFSCMVGHEALPLAFTQKTISLSPGKPTHVNVSVVMAEVDGT

SEQ ID NO: 74 - protein, 467 aa, synthetic construct; identical to SEQ ID NO: 71

SEQ ID NO: 75 - protein, 214 aa, synthetic construct; identical to SEQ ID NO: 60

SEQ ID NO: 76 - protein, 490 aa, synthetic construct
EIVLTQSPATLSLSPGERATLSCRASQSVSSYLAWYQQKPGQAPRLLIYDASNRATGIPARFSGSGSGTDFTLTISSLEPEDFAVYYCQQRSNWPPSTFGQGTRLEIKGGGGSGGGGSGGGGSGGGGSEVQLLESGGGLVQPGGSLRLSCAASGFTFTSYAMSWVRQAPGKGLEWVSTISGSGGGTYYTDSVKGRFTISRDNSKNTLYLQMNSLRAEDTAVYYCAQGSSIFDYWGQGTLVTVSSVPSTPPTPSPSTPPTPSPSCCHPRLSLHRPALEDLLLGSEANLTCTLTGLRDASGVTFTWTPSSGKSAVQGPPERDLCGCYSVSSVLPGCAEPWNHGKTFTCTAAYPESKTPLTATLSKSGQPFRPEVHLLPPSREEMTKNQVSLTCLARGFYPKDVLVRWLSNSQEENNYKTTPSRQEPSQGTTTFAVTSKLTVDKSRWQQGNVFSCMVGHEALPLAFTQKTISLSPGKPTHVNVSVVMAEVDGT

SEQ ID NO: 77 - protein, 467 aa, synthetic construct; identical to SEQ ID NO: 71

SEQ ID NO: 78 - protein, 214 aa, synthetic construct; identical to SEQ ID NO: 60

SEQ ID NO: 79 - protein, 457 aa, synthetic construct
EVQLVQSGAEVKKPGASVKVSCKASGFSLTNYGVHWMRQAPGQGLEWIGVIWSGGNTDYNTPFTSRVTITSDKSTSTAYMELSSLRSEDTAVYYCARALTYYDYEFAYWGQGTLVTVSSASPTSPKVFPLSLDSTPQDGNVVVACLVQGFFPQEPLSVTWSESGQNVTARNFPPSQDASGDLYTTSSQLTLPATQCPDGKSVTCHVKHYTNPSQDVTVPCRVPPPPPCCHPRLSLHRPALEDLLLGSEANLTCTLTGLRDASGATFTWTPSSGKSAVQGPPERDLCGCYSVSSVLPGCAQPWNHGETFTCTAAHPELKTPLTANITKSGNTFRPEVHLLPPPSEELALNELVTLTCLARGFSPKDVLVRWLQGSQELPREKYLTWASRQEPSQGTTTFAVTSILRVAAEDWKKGETFSCMVGHEALPLAFTQKTIDRLAGKPTHVNVSVVMAEVDGT

SEQ ID NO: 80 - protein, 214 aa, synthetic construct; identical to SEQ ID NO: 60

SEQ ID NO: 81 - protein, 477 aa, synthetic construct
EIVLTQSPATLSLSPGERATLSCRASQSVSSYLAWYQQKPGQAPRLLIYDASNRATGIPARFSGSGSGTDFTLTISSLEPEDFAVYYCQQRSNWPPSTFGQGTRLEIKGGGGSGGGGSGGGGSGGGGSEVQLLESGGGLVQPGGSLRLSCAASGFTFTSYAMSWVRQAPGKGLEWVSTISGSGGGTYYTDSVKGRFTISRDNSKNTLYLQMNSLRAEDTAVYYCAQGSSIFDYWGQGTLVTVSSVPPPPPCCHPRLSLHRPALEDLLLGSEANLTCTLTGLRDASGATFTWTPSSGKSAVQGPPERDLCGCYSVSSVLPGCAQPWNHGETFTCTAAHPELKTPLTANITKSGQPFRPEVHLLPPSREEMTKNQVSLTCLARGFYPKDIAVEWESNGQPENNYKTTPSRQEPSQGTTTFAVTSKLTVDKSRWQQGNVFSCSVMHEALHNHYTQKTISLSPGKPTHVNVSVVMAEVDGT

SEQ ID NO: 82 - protein, 454 aa, synthetic construct
EVQLVQSGAEVKKPGASVKVSCKASGFSLTNYGVHWMRQAPGQGLEWIGVIWSGGNTDYNTPFTSRVTITSDKSTSTAYMELSSLRSEDTAVYYCARALTYYDYEFAYWGQGTLVTVSSASPTSPKVFPLSLDSTPQDGNVVVACLVQGFFPQEPLSVTWSESGQNVTARNFPPSQDASGDLYTTSSQLTLPATQCPDGKSVTCHVKHYTNPSQDVTVPCRVPPPPPCCHPRLSLHRPALEDLLLGSEANLTCTLTGLRDASGATFTWTPSSGKSAVQGPPERDLCGCYSVSSVLPGCAQPWNHGETFTCTAAHPELKTPLTANITKSGQPREPQVYTLPPPSEELALNELVTLTCLVKGFYPSDIAVEWLQGSQELPREKYLTWAPVLDSDGSFFLYSILRVAAEDWKKGDTFSCSVMHEALHNHYTQKSLDRSPGKPTHVNVSVVMAEVDGT

SEQ ID NO: 83 - protein, 214 aa, synthetic construct; identical to SEQ ID NO: 60

SEQ ID NO: 84 - protein, 477 aa, synthetic construct
EIVLTQSPATLSLSPGERATLSCRASQSVSSYLAWYQQKPGQAPRLLIYDASNRATGIPARFSGSGSGTDFTLTISSLEPEDFAVYYCQQRSNWPPSTFGQGTRLEIKGGGGSGGGGSGGGGSGGGGSEVQLLESGGGLVQPGGSLRLSCAASGFTFTSYAMSWVRQAPGKGLEWVSTISGSGGGTYYTDSVKGRFTISRDNSKNTLYLQMNSLRAEDTAVYYCAQGSSIFDYWGQGTLVTVSSVPPPPPCCHPRLSLHRPALEDLLLGSEANLTCTLTGLRDASGATFTWTPSSGKSAVQGPPERDLCGCYSVSSVLPGCAQPWNHGETFTCTAAHPELKTPLTANITKSGQPFRPEVHLLPPSREEMTKNQVSLTCLARGFYPKDIAVRWLSNSQEENNYKTTPSRQEPSQGTTTFAVTSKLTVDKSRWQQGNVFSCMVGHEALPLAFTQKTISLSPGKPTHVNVSVVMAEVDGT

SEQ ID NO: 85 - protein, 454 aa, synthetic construct
EVQLVQSGAEVKKPGASVKVSCKASGFSLTNYGVHWMRQAPGQGLEWIGVIWSGGNTDYNTPFTSRVTITSDKSTSTAYMELSSLRSEDTAVYYCARALTYYDYEFAYWGQGTLVTVSSASPTSPKVFPLSLDSTPQDGNVVVACLVQGFFPQEPLSVTWSESGQNVTARNFPPSQDASGDLYTTSSQLTLPATQCPDGKSVTCHVKHYTNPSQDVTVPCRVPPPPPCCHPRLSLHRPALEDLLLGSEANLTCTLTGLRDASGATFTWTPSSGKSAVQGPPERDLCGCYSVSSVLPGCAQPWNHGETFTCTAAHPELKTPLTANITKSGQPREPQVYTLPPPSEELALNELVTLTCLVKGFYPSDVLVRWLQGSQELPREKYLTWAPVLDSDGSFFLYSILRVAAEDWKKGDTFSCMVGHEALPLAFTQKSLDRSPGKPTHVNVSVVMAEVDGT

SEQ ID NO: 86 - protein, 214 aa, synthetic construct; identical to SEQ ID NO: 60

SEQ ID NO: 87 - protein, 471 aa, synthetic construct
EVQLVESGGGLVQPGGSLRLSCAASGFNIKDTYIHWVRQAPGKGLEWVARIYPTNGYTRYADSVKGRFTISADTSKNTAYLQMNSLRAEDTAVYYCSRWGGDGFYAMDYWGQGTLVTVSSASPTSPKVFPLSLCSTQPDGNVVIACLVQGFFPQEPLSVTWSESGQGVTARNFPPSQDASGDLYTTSSQLTLPATQCLAGKSVTCHVKHYTNPSQDVTVPCPVPSTPPTPSPSTPPTPSPSCCHPRLSLHRPALEDLLLGSEANLTCTLTGLRDASGVTFTWTPSSGKSAVQGPPERDLCGCYSVSSVLPGCAEPWNHGKTFTCTAAYPESKTPLTATLSKSGNTFRPEVHLLPPPSEELALNELVTLTCLARGFSPKDVLVRWLQGSQELPREKYLTWASRQEPSQGTTTFAVTSILRVAAEDWKKGETFSCMVGHEALPLAFTQKTIDRLAGKPTHVNVSVVMAEVDGT

SEQ ID NO: 88 - protein, 214 aa, synthetic construct
DIQMTQSPSSLSASVGDRVTITCRASQDVNTAVAWYQQKPGKAPKLLIYSASFLYSGVPSRFSGSRSGTDFTLTISSLQPEDFATYYCQQHYTTPPTFGQGTKVEIKRTVAAPSVFIFPPSDEQLKSGTASVVCLLNNFYPREAKVQWKVDNALQSGNSQESVTEQDSKDSTYSLSSTLTLSKADYEKHKVYACEVTHQGLSSPVTKSFNRGEC

SEQ ID NO: 89 - protein, 4 aa, synthetic construct
PLAF

SEQ ID NO: 90 - protein, 4 aa, synthetic construct
HNHY

SEQ ID NO: 91 - protein, 113 aa, synthetic construct
GNTFRPEVHLLPPPSEELALNELVTLTCLARGFSPKDVLVRWLQGSQELPREKYLTWASRQEPSQGTTTFAVTSILRVAAEDWKKGETFSCMVGHEALPLAFTQKTIDRLAGK

SEQ ID NO: 92 - protein, 110 aa, synthetic construct
GQPFRPEVHLLPPSREEMTKNQVSLTCLARGFYPKDIAVEWESNGQPENNYKTTPSRQEPSQGTTTFAVTSKLTVDKSRWQQGNVFSCSVMHEALHNHYTQKTISLSPGK

SEQ ID NO: 93 - protein, 110 aa, synthetic construct
GQPREPQVYTLPPPSEELALNELVTLTCLVKGFYPSDIAVEWLQGSQELPREKYLTWAPVLDSDGSFFLYSILRVAAEDWKKGDTFSCSVMHEALHNHYTQKSLDRSPGK

SEQ ID NO: 94 - protein, 107 aa, synthetic construct
GQPREPQVYTLPPSREEMTKNQVSLTCLVKGFYPSDIAVEWESNGQPENNYKTTPPVLDSDGSFFLYSKLTVDKSRWQQGNVFSCSVMHEALHNHYTQKSLSLSPGK

SEQ ID NO: 95 - protein, 11 aa, synthetic construct
ANLTCTLTGLR

SEQ ID NO: 96 - protein, 16 aa, synthetic construct
LAGKPTHVNVSVVMAE

SEQ ID NO: 97 - protein, 16 aa, synthetic construct
SPGKPTHVNVSVVMAE

SEQ ID NO: 98 - protein, 20 aa, synthetic construct
TISLSPGKPTHVNVSVVMAE

SEQ ID NO: 99 - protein, 11 aa, synthetic construct
ANLTCTLTGLR

SEQ ID NO: 100 - protein, 9 aa, synthetic construct
TPLTANITK

SEQ ID NO: 101 - protein, 16 aa, synthetic construct
LAGKPTHVNVSVVMAE

SEQ ID NO: 102 - protein, 20 aa, synthetic construct
TISLSPGKPTHVNVSVVMAE

SEQ ID NO: 103 - protein, 16 aa, synthetic construct
SPGKPTHVNVSVVMAE